European Patent Application EP 4 796 641 A1, published August 26, 2026. Title: 一种用于清除乙肝病毒的病毒基因治疗载体及应用. Applicant: 哈尔滨工业大学. The sequence listing filed with the application follows.

SEQUENCE LISTING (25 sequences)

SEQ ID NO: 1 - DNA, 800 bp, synthetic construct
  source 1..800: mol_type = other DNA
gtggcgcatgcctgtaacctgagctacttggtaggctgaggcagggaggcaggagaattgcttgaatctgggaggtggaggttgtagtgagctgagatcgtgccattgcactccagcctgggtgacagagcgagactccgtctcaaaaaaaaaaaaagttattgatgacttagattttcaacactgccttaaattttgcggcaaagaggatgcctcaacctagtccctgcctcagcccacaaccttcatatggttctaccaggcaaagctcctatccccaaatcctgggaaacgagcttggaggaggacattgtctcttactcccatgggaagtgtcccccattcactctatcacttagcaccctacatcctgagcttccactatgtgcccagcttttttctgggaggtccccagaaagaggacacctgaggaggccccaggggtggcccccaggggaatcccaggcctggctcaggctggacattcccaggcctgccctggctgagtctccagctggtgggtctcctggaaactccccgggctggttttgaggtgggagccccacagggaagcaatttacatacacaacagcccagtcatgtcaacctgccccatctgatgccagaataaaggggagatgggtccattctgcaggtctcagtcatgggcacccggagaagaggaaggacatttcactgtcagcccaggtgagtccagaagccagctcctggaacaatgccagggtcctgaacactcaagctcaacccctgctctcagctactgctggtggcttgaaatc

SEQ ID NO: 2 - DNA, 304 bp, synthetic construct
  source 1..304: mol_type = other DNA
cgttacataacttacggtaaatggcccgcctggctgaccgcccaacgacccccgcccattgacgtcaataatgacgtatgttcccatagtaacgtcaatagggactttccattgacgtcaatgggtggagtatttacggtaaactgcccacttggcagtacatcaagtgtatcatatgccaagtacgccccctattgacgtcaatgacggtaaatggcccgcctggcattatgcccagtacatgaccttatgggactttcctacttggcagtacatctacgtattagtcatcgctattaccatg

SEQ ID NO: 3 - DNA, 107 bp, synthetic construct
  source 1..107: mol_type = other DNA
tcctgcccaaggtcttacataagaggactcttggactcccagcaatgtcaacgaccgaccttgaggcctacttcaaagactgtgtgtttaaggactgggaggagctg

SEQ ID NO: 4 - DNA, 81 bp, synthetic construct
  source 1..81: mol_type = other DNA
aagccaagacctgccaggagtgtctctaagagatccaggagggagccacccccaaggaccctgccagccacagacctccaa

SEQ ID NO: 5 - DNA, 507 bp, synthetic construct
  source 1..507: mol_type = other DNA
aagtccccaccgaccatggtggacagcctcctggcagtcaccctggctggaaacctgggcctgaccttcctccgaggttcccagacccagagccatccagacctgggaactgagggctgctgggaccagctctctgcccctcggacctttacgcttttggaccccaaggcatctctgttaaccatggccttcctcaatggcgccctggatggggtcatccttggagactacctgagccggactcctgagccccggccatccctcagccacttgctgagccagtactatggggctggggtggccagagacccagggttccgcagcaacttccgacggcagaacggtgctgctctgacttcagcctccatcctggcccagcaggtgtggggaacccttgtccttctacagaggctggagccagtacacctccagcttcagtgcatgagccaagaacagctggcccaggtggctgccaatgctaccaaggaattcactgaggccttcctg

SEQ ID NO: 6 - DNA, 63 bp, synthetic construct
  source 1..63: mol_type = other DNA
atggcccagggtgtcctctggatcctactcggattgctactgtggtcagacccagggacagcc

SEQ ID NO: 7 - DNA, 438 bp, synthetic construct
  source 1..438: mol_type = other DNA
ccggccatccacccccgctgccgctggggagcggcgccttatcggggccgcccgaagctgctgcagctgccgctgggattcttgtacgtgcatcacacctacgtgcctgcaccaccctgcacggacttcacgcgctgcgcagccaacatgcgctccatgcagcgctaccaccaggacacgcaaggctggggagacatcggctacagtttcgtggtgggctcggacggctacgtgtacgagggacgcggctggcactgggtgggcgcccacacgctcggccacaactcccggggcttcggcgtggccatagtgggcaactacaccgcggcgctgcccaccgaggccgctctgcgcacggtgcgcgacacgctcccgagttgtgcggtgcgcgccggcctcctgcggccagactacgcgctgctgggccaccgccagctg

SEQ ID NO: 8 - DNA, 836 bp, synthetic construct
  source 1..836: mol_type = other DNA
gtaagtatcaaggttacaagacaggtttaaggagaccaatagaaactgggcttgtcgagacagagaagactcttgcgtttctgataggcacctattggtcttactgacatccactttgcctttctctccacaggtgtccactcccagttcaattacagctcttaaggctagagtacttaatacgactcactataggctagcctcgagaattcacgcgtcgagcatgcatctagggcggccaattccgcccctctcccccccccccctctccctcccccccccctaacgttactggccgaagccgcttggaataaggccggtgtgcgtttgtctatatgttattttccaccatattgccgtcttttggcaatgtgagggcccggaaacctggccctgtcttcttgacgagcattcctaggggtctttcccctctcgccaaaggaatgcaaggtctgttgaatgtcgtgaaggaagcagttcctctggaagcttcttgaagacaaacaacgtctgtagcgaccctttgcaggcagcggaaccccccacctggcgacaggtgcctctgcggccaaaagccacgtgtataagatacacctgcaaaggcggcacaaccccagtgccacgttgtgagttggatagttgtggaaagagtcaaatggctctcctcaagcgtattcaacaaggggctgaaggatgcccagaaggtaccccattgtatgggatctgatctggggcctcggtgcacatgctttacatgtgtttagtcgaggttaaaaaaacgtctaggccccccgaaccacggggacgtggttttcctttgaaaaacacgatgataa

SEQ ID NO: 9 - DNA, 1653 bp, synthetic construct
  source 1..1653: mol_type = other DNA
atggaagacgccaaaaacataaagaaaggcccggcgccattctatccgctggaagatggaaccgctggagagcaactgcataaggctatgaagagatacgccctggttcctggaacaattgcttttacagatgcacatatcgaggtggacatcacttacgctgagtacttcgaaatgtccgttcggttggcagaagctatgaaacgatatgggctgaatacaaatcacagaatcgtcgtatgcagtgaaaactctcttcaattctttatgccggtgttgggcgcgttatttatcggagttgcagttgcgcccgcgaacgacatttataatgaacgtgaattgctcaacagtatgggcatttcgcagcctaccgtggtgttcgtttccaaaaaggggttgcaaaaaattttgaacgtgcaaaaaaagctcccaatcatccaaaaaattattatcatggattctaaaacggattaccagggatttcagtcgatgtacacgttcgtcacatctcatctacctcccggttttaatgaatacgattttgtgccagagtccttcgatagggacaagacaattgcactgatcatgaactcctctggatctactggtctgcctaaaggtgtcgctctgcctcatagaactgcctgcgtgagattctcgcatgccagagatcctatttttggcaatcaaatcattccggatactgcgattttaagtgttgttccattccatcacggttttggaatgtttactacactcggatatttgatatgtggatttcgagtcgtcttaatgtatagatttgaagaagagctgtttctgaggagccttcaggattacaagattcaaagtgcgctgctggtgccaaccctattctccttcttcgccaaaagcactctgattgacaaatacgatttatctaatttacacgaaattgcttctggtggcgctcccctctctaaggaagtcggggaagcggttgccaagaggttccatctgccaggtatcaggcaaggatatgggctcactgagactacatcagctattctgattacacccgagggggatgataaaccgggcgcggtcggtaaagttgttccattttttgaagcgaaggttgtggatctggataccgggaaaacgctgggcgttaatcaaagaggcgaactgtgtgtgagaggtcctatgattatgtccggttatgtaaacaatccggaagcgaccaacgccttgattgacaaggatggatggctacattctggagacatagcttactgggacgaagacgaacacttcttcatcgttgaccgcctgaagtctctgattaagtacaaaggctatcaggtggctcccgctgaattggaatccatcttgctccaacaccccaacatcttcgacgcaggtgtcgcaggtcttcccgacgatgacgccggtgaacttcccgccgccgttgttgttttggagcacggaaagacgatgacggaaaaagagatcgtggattacgtcgccagtcaagtaacaaccgcgaaaaagttgcgcggaggagttgtgtttgtggacgaagtaccgaaaggtcttaccggaaaactcgacgcaagaaaaatcagagagatcctcataaaggccaagaagggcggaaagatcgccgtgtaa

SEQ ID NO: 10 - DNA, 37 bp, synthetic construct
  source 1..37: mol_type = other DNA
cgggatcccgatggaagacgccaaaaacataaagaaa

SEQ ID NO: 11 - DNA, 35 bp, synthetic construct
  source 1..35: mol_type = other DNA
ccaagcttggttacacggcgatctttccgcccttc

SEQ ID NO: 12 - DNA, 32 bp, synthetic construct
  source 1..32: mol_type = other DNA
cgacgcgtcggtggcgcatgcctgtaacctga

SEQ ID NO: 13 - DNA, 39 bp, synthetic construct
  source 1..39: mol_type = other DNA
catgccatggcatggatttcaagccaccagcagtagctg

SEQ ID NO: 14 - DNA, 32 bp, synthetic construct
  source 1..32: mol_type = other DNA
cgacgcgtcgtcctgcccaaggtcttacataa

SEQ ID NO: 15 - DNA, 30 bp, synthetic construct
  source 1..30: mol_type = other DNA
cgagctcgcagctcctcccagtccttaaac

SEQ ID NO: 16 - DNA, 21 bp, synthetic construct
  source 1..21: mol_type = other DNA
gatgagcacttttaaagttct

SEQ ID NO: 17 - DNA, 19 bp, synthetic construct
  source 1..19: mol_type = other DNA
gttgtcagaagtaagttgg

SEQ ID NO: 18 - DNA, 30 bp, synthetic construct
  source 1..30: mol_type = other DNA
ccatcgatggatgaaatccccccctaccat

SEQ ID NO: 19 - DNA, 32 bp, synthetic construct
  source 1..32: mol_type = other DNA
cgggatcccgttacttgtcatcgtcatccttg

SEQ ID NO: 20 - DNA, 33 bp, synthetic construct
  source 1..33: mol_type = other DNA
cgggatcccggtaagtatcaaggttacaagaca

SEQ ID NO: 21 - DNA, 54 bp, synthetic construct
  source 1..54: mol_type = other DNA
acgcgtcgacgtcggccatagcggccgcggaattatcatcgtgtttttcaaagg

SEQ ID NO: 22 - DNA, 56 bp, synthetic construct
  source 1..56: mol_type = other DNA
acgcgtcgacgtcggccatagcggccgcggaaatggcccagggcgtgctctggatt

SEQ ID NO: 23 - DNA, 32 bp, synthetic construct
  source 1..32: mol_type = other DNA
gaagatcttcttacttgtcatcgtcatccttg

SEQ ID NO: 24 - DNA, 20 bp, synthetic construct
  source 1..20: mol_type = other DNA
gtctgtgccttctcatctgc

SEQ ID NO: 25 - DNA, 22 bp, synthetic construct
  source 1..22: mol_type = other DNA
acaagagatgattaggcagagg